European Patent Application EP 4 198 143 A1, published June 21, 2023. Title: Modified primers for loop-mediated isothermal amplification and use thereof. Applicant: 주식회사 원드롭. The sequence listing filed with the application follows.

SEQUENCE LISTING (18 sequences)

SEQ ID NO: 1 - DNA, 19 bp, synthetic construct
  source 1..19: mol_type = other DNA
tggctactaccgaagagct

SEQ ID NO: 2 - DNA, 20 bp, synthetic construct
  misc_feature 1..20: note = DNA
  source 1..20: mol_type = other DNA
tgcagcattgttagcaggat

SEQ ID NO: 3 - DNA, 41 bp, synthetic construct
  misc_feature 1..41: note = DNA
  source 1..41: mol_type = other DNA
tctggcccagttcctaggtagtgacgaattcgtggtggtga

SEQ ID NO: 4 - DNA, 40 bp, synthetic construct
  misc_feature 1..40: note = DNA
  source 1..40: mol_type = other DNA
agacggcatcatatgggttgcacgggtgccaatgtgatct

SEQ ID NO: 5 - DNA, 24 bp, synthetic construct
  misc_feature 1..24: note = DNA
  source 1..24: mol_type = other DNA
gaaataccatcttggactgagatc

SEQ ID NO: 6 - DNA, 20 bp, synthetic construct
  misc_feature 1..20: note = DNA
  source 1..20: mol_type = other DNA
tgagggagccttgaatacac

SEQ ID NO: 7 - DNA, 48 bp, synthetic construct
  source 1..48: mol_type = other DNA
  misc_feature 1..41: note = DNA
  misc_feature 42..44: note = RNA
  misc_feature 45..48: note = DNA
tctggcccagttcctaggtagtgacgaattcgtggtggtgacggtaaa

SEQ ID NO: 8 - DNA, 47 bp, synthetic construct
  misc_feature 1..40: note = DNA
  misc_feature 41..43: note = RNA
  misc_feature 44..47: note = DNA
  source 1..47: mol_type = other DNA
agacggcatcatatgggttgcacgggtgccaatgtgatcttttggtg

SEQ ID NO: 9 - DNA, 20 bp, synthetic construct
  misc_feature 1..20: note = DNA
  source 1..20: mol_type = other DNA
ccactagaggagctactgta

SEQ ID NO: 10 - DNA, 18 bp, synthetic construct
  misc_feature 1..18: note = DNA
  source 1..18: mol_type = other DNA
tgacaagctacaacacgt

SEQ ID NO: 11 - DNA, 48 bp, synthetic construct
  misc_feature 1..48: note = DNA
  source 1..48: mol_type = other DNA
aggtgagggttttctacatcactatattggaacaagcaaattctatgg

SEQ ID NO: 12 - DNA, 43 bp, synthetic construct
  misc_feature 1..43: note = DNA
  source 1..43: mol_type = other DNA
atgggttgggattatcctaaatgtgtgcgagcaagaacaagtg

SEQ ID NO: 13 - DNA, 25 bp, synthetic construct
  source 1..25: mol_type = other DNA
cagtttttaacatgttgtgccaacc

SEQ ID NO: 14 - DNA, 19 bp, synthetic construct
  misc_feature 1..19: note = DNA
  source 1..19: mol_type = other DNA
gagccatgcctaacatgct

SEQ ID NO: 15 - DNA, 48 bp, synthetic construct; identical to SEQ ID NO: 7
  misc_feature 1..41: note = DNA
  misc_feature 42..44: note = RNA
  misc_feature 45..48: note = DNA
  source 1..48: mol_type = other DNA
  misc_feature 30: note = internal dT

SEQ ID NO: 16 - DNA, 47 bp, synthetic construct; identical to SEQ ID NO: 8
  misc_feature 1..40: note = DNA
  misc_feature 41..43: note = RNA
  misc_feature 44..47: note = DNA
  source 1..47: mol_type = other DNA
  misc_feature 27: note = Internal dT

SEQ ID NO: 17 - DNA, 55 bp, synthetic construct
  misc_feature 1..48: note = DNA
  misc_feature 49..51: note = RNA
  misc_feature 52..55: note = DNA
  source 1..55: mol_type = other DNA
  misc_feature 28: note = internal dT
aggtgagggttttctacatcactatattggaacaagcaaattctatggtggttgg

SEQ ID NO: 18 - DNA, 50 bp, synthetic construct
  misc_feature 1..43: note = DNA
  misc_feature 44..46: note = RNA
  misc_feature 47..50: note = DNA
  source 1..50: mol_type = other DNA
  misc_feature 26: note = internal dT
atgggttgggattatcctaaatgtgtgcgagcaagaacaagtgaggccat